European Patent Application EP 4 134 377 A1, published February 15, 2023. Title: PD-1 VARIANTS WITH INCREASED BINDING TO PD-L1. Applicant: Korea University Research and Business Foundation. The sequence listing filed with the application follows.

SEQUENCE LISTING (11 sequences)

SEQ ID NO: 1 - protein, 143 aa, Artificial Sequence
  WT PD-1
LDSPDRPWNPPTFSPALLVVTEGDNATFTCSFSNTSESFVLNWYRMSPSNQTDKLAAFPEDRSQPGQDCRFRVTQLPNGRDFHMSVVRARRNDSGTYLCGAISLAPKAQIKESLRAELRVTERRAEVPTAHPSPSPRPAGQFQ

SEQ ID NO: 2 - protein, 143 aa, Artificial Sequence
  N-IITV
LDSPDRPWNPPTISPALLVVTEGDNATFTCSFSNTSESFVLNWYRISPSNQTDKLAAFPEDRSQPGQDTRFRVTQLPNGRDFHMSVVRARRNDSGTYLCVAISLAPKAQIKESLRAELRVTERRAEVPTAHPSPSPRPAGQFQ

SEQ ID NO: 3 - protein, 143 aa, Artificial Sequence
  Q_IITV
LDSPDRPWNPPTISPALLVVTEGDQATFTCSFSQTSESFVLNWYRISPSQQTDKLAAFPEDRSQPGQDTRFRVTQLPNGRDFHMSVVRARRQDSGTYLCVAISLAPKAQIKESLRAELRVTERRAEVPTAHPSPSPRPAGQFQ

SEQ ID NO: 4 - protein, 143 aa, Artificial Sequence
  JY_Q10
LDSPDRPWNPPTISPALLVVTEGDQATFTCSLSQTSESFVLNWYRISPSQQMDKLAAFPEDRSQPGQDTRFRVTQLPNGRDFHMSVDRARRQDSGSYLCVAISLAPKVQIKESLRAELRVTERRAEVPTAHPSPSPRPAGQFQ

SEQ ID NO: 5 - protein, 143 aa, Artificial Sequence
  JY_Q12
LDSPDRPLDPPTISPALLVVTEGDQATFTCSFSQTSKSFVLNWYRISPSQQTDKLAAFPEDRSQPGQDTRFRVTQLPNGRDFHMSVVRARRQDSGTYLCVAISLAPKVQIKESLRAELRVTERRAEVPTAHPSPSPRPACQFQ

SEQ ID NO: 6 - protein, 143 aa, Artificial Sequence
  JY_Q18
LDSPDRPWNPPTISPALLVVTEGDQATFTCGLPQTSESFVLNWYRIGPSQQMDKLAAFPEDRSQPGQDTRFRVTQLPNGRDFHMSVVRARRQDSGTYLCVAISLAPKVQIKESLRAELRVTERRAEVRTAHPSPSPRSAGQFQ

SEQ ID NO: 7 - protein, 143 aa, Artificial Sequence
  JY_Q33
LDSPDRPWNPPTISPALLVVTEGDQATFTCSFSRTSESFVLNWYRISPSQQTDKLAAFPEDRSQPGQDTRFRVTQLPNGRDFHMSVVGAQRQDSGTYLCVAISLAPKVQIKESLRAELRVTERRAEVPTAHPSPSPRPAGQFQ

SEQ ID NO: 8 - protein, 143 aa, Artificial Sequence
  JY_Q12-1
LDSPDRPLDPPTISPALLVVTEGDNATFTCSFSQTSKSFVLNWYRISPSQQTDKLAAFPEDRSQPGQDTRFRVTQLPNGRDFHMSVVRARRQDSGTYLCVAISLAPKVQIKESLRAELRVTERRAEVPTAHPSPSPRPACQFQ

SEQ ID NO: 9 - protein, 143 aa, Artificial Sequence
  JY_Q12-2
LDSPDRPLDPPTISPALLVVTEGDQATFTCSFSNTSKSFVLNWYRISPSQQTDKLAAFPEDRSQPGQDTRFRVTQLPNGRDFHMSVVRARRQDSGTYLCVAISLAPKVQIKESLRAELRVTERRAEVPTAHPSPSPRPACQFQ

SEQ ID NO: 10 - protein, 143 aa, Artificial Sequence
  JY_Q12-3
LDSPDRPLDPPTISPALLVVTEGDQATFTCSFSQTSKSFVLNWYRISPSNQTDKLAAFPEDRSQPGQDTRFRVTQLPNGRDFHMSVVRARRQDSGTYLCVAISLAPKVQIKESLRAELRVTERRAEVPTAHPSPSPRPACQFQ

SEQ ID NO: 11 - protein, 143 aa, Artificial Sequence
  JY_Q12-4
LDSPDRPLDPPTISPALLVVTEGDQATFTCSFSQTSKSFVLNWYRISPSQQTDKLAAFPEDRSQPGQDTRFRVTQLPNGRDFHMSVVRARRNDSGTYLCVAISLAPKVQIKESLRAELRVTERRAEVPTAHPSPSPRPACQFQ